European Patent Specification EP 3 386 558 B1, published October 4, 2023. Title: POLY(ESTER UREA) FIBER DEVICES AND RELATED METHODS. Applicant: COOK BIOTECH INCORPORATED Wade, Mary Patel, Umesh Shah, Bhavin. The sequence listing filed with the application follows.

SEQUENCE LISTING (4 sequences)

SEQ ID NO: 1 - protein, 7 aa, Artificial Sequence
  Synthetic Construct
GGGKRSR

SEQ ID NO: 2 - protein, 5 aa, Artificial Sequence
  Synthetic Construct
GRGDS

SEQ ID NO: 3 - protein, 5 aa, Artificial Sequence
  Synthetic Construct
YGFGG

SEQ ID NO: 4 - protein, 20 aa, Artificial Sequence
  Synthetic Construct
KIPKASSVPTELSAISTLYL